European Patent Application EP 4 481 384 A1, published December 25, 2024. Title: NON-SPECIFIC REACTION INHIBITOR. Applicant: LSI Medience Corporation. The sequence listing filed with the application follows.

SEQUENCE LISTING (2 sequences)

SEQ ID NO: 1 - protein, 13 aa, synthetic construct
  REGION 1..13: note = human IgG binding peptide
DCAWHLGELVWCT

SEQ ID NO: 2 - protein, 16 aa, synthetic construct
  REGION 1..16: note = human IgA binding peptide
HMVCLSYRGRPVCFSL